European Patent Specification EP 4 117 445 B1, published February 11, 2026. Title: LACTOSE REDUCED DAIRY POWDER. Applicant: DSM IP Assets B.V. The sequence listing filed with the application follows.

SEQUENCE LISTING (7 sequences)

SEQ ID NO: 1 - protein, 594 aa, Sporobolomyces singularis
  Beta-hexosyltransferase of organism Sporobolomyces singularis (also referred to as BHT-132, wildtype)
MMLHAALLVALPCVVLARPAGAVTYPGAIPLSLTSNYETPSPTAIPLEPTPTATGTAELDALWNLVEAQYPVQTAAVTTLVTVPDDYKFEADPPSYALAGYETSEIAGLKFPKGFKFGVAGAAIQVEGAAKAEGRGPSTWDYLCHHYASTQCNNYDPDITTNHYYLYPLDFARLQHLGINTYSFSISWTRIYPLGAGYVNEAGLAHYDAVIHSAKKYGLEPVGTVFHWDTPLSLMLKYGAWQDTGDQIVKDFVTYATTVFKRYGNEVKTWFTFNEPRVFCSQNSGLPYNLTYPEGINSTSAVFRCTYNVLKAHGHAVKVYRDLVASGTIAAGEIGFKSDDNYPIPARPGNADDEESAKRHEAFRIGIFAQPVYGNGDYPDVVKETVGDMLPALTDEDKGYIKGSGDIFAIDGYRTDISHAALNGIANCIRNQSDPNWPVCEEGSDPFAHVYPSGFAIGQSADPLSSWLVNSAPFIRDQLKFLTQTYPAKGGIYFSEFGWAEDAEYDRQLLYQITWDGLRTQYLTDYLSQLLLAVHKDGINLRGALTWSFVDNWEWGLGMQQKFGFQFVNQSDPDLTRTFKLSAHAYAQFGRNHL

SEQ ID NO: 2 - protein, 557 aa, Artificial Sequence
  sets out the sequence of BHT-134 which is a deletion mutant derived from SEQ ID NO: 1 and the deletion starts at position 18 up to and including position 54
MMLHAALLVALPCVVLAGTAELDALWNLVEAQYPVQTAAVTTLVTVPDDYKFEADPPSYALAGYETSEIAGLKFPKGFKFGVAGAAIQVEGAAKAEGRGPSTWDYLCHHYASTQCNNYDPDITTNHYYLYPLDFARLQHLGINTYSFSISWTRIYPLGAGYVNEAGLAHYDAVIHSAKKYGLEPVGTVFHWDTPLSLMLKYGAWQDTGDQIVKDFVTYATTVFKRYGNEVKTWFTFNEPRVFCSQNSGLPYNLTYPEGINSTSAVFRCTYNVLKAHGHAVKVYRDLVASGTIAAGEIGFKSDDNYPIPARPGNADDEESAKRHEAFRIGIFAQPVYGNGDYPDVVKETVGDMLPALTDEDKGYIKGSGDIFAIDGYRTDISHAALNGIANCIRNQSDPNWPVCEEGSDPFAHVYPSGFAIGQSADPLSSWLVNSAPFIRDQLKFLTQTYPAKGGIYFSEFGWAEDAEYDRQLLYQITWDGLRTQYLTDYLSQLLLAVHKDGINLRGALTWSFVDNWEWGLGMQQKFGFQFVNQSDPDLTRTFKLSAHAYAQFGRNHL

SEQ ID NO: 3 - DNA, 1782 bp, Artificial Sequence
  sets out a codon-adapted DNA sequence for expression of SEQ ID NO: 1 in Aspergillus niger
atgatgcttcacgctgctctccttgttgctcttccttgcgttgtccttgctcgtcccgccggtgctgtcacctaccccggtgccatccccctctccctcacctcgaactacgagactcccagccctactgccattcctctggagcccacccccactgccactggtactgctgagctcgatgccctctggaacttggttgaggctcagtaccccgtgcagactgctgccgtcaccaccctcgtcaccgttcccgatgactacaagttcgaggccgatcctcctagctacgctcttgctggatacgagacttctgagattgctggtctgaagttccccaagggcttcaagttcggtgttgctggtgccgccatccaggttgagggtgctgccaaggccgagggccgtggtccctccacctgggactacctctgccaccactacgcctccacccagtgcaacaactacgaccctgacatcaccaccaaccactactacctctaccccctcgacttcgctcgtctgcagcacctgggtatcaacacctactctttctccatctcctggactcgcatctaccctcttggtgctggctacgtcaacgaggctggtctggctcactacgatgccgtcatccactctgccaagaagtacggcttggagcctgttggtaccgtcttccactgggatactcctctgagcttgatgctcaagtacggtgcctggcaggacaccggtgaccagattgtcaaggacttcgtcacctacgccaccactgtcttcaagcgctacggcaacgaggtcaagacctggttcaccttcaacgagcctcgtgtcttctgctctcagaactccggtctgccctacaacctgacctacccagaaggcatcaactccacctcggcggtgttccgctgcacctacaacgtcctcaaggcccacggccacgccgtcaaggtctaccgtgatcttgttgcctccggtaccattgctgctggtgagatcggtttcaagtccgacgacaactaccccatccccgctcgccccggcaacgccgatgatgaggagtccgccaagcgtcacgaagcgttccgtatcggtatcttcgctcagcccgtgtatggcaacggtgactaccccgatgtcgtcaaggagactgttggtgacatgcttcccgccctcaccgacgaggacaagggctacatcaagggctccggtgacatcttcgccattgacggctaccgcactgatatatctcacgctgccctcaacggcattgccaactgcattcgcaaccagtccgaccccaactggcccgtctgcgaagaaggaagcgaccccttcgctcacgtctacccctccggattcgccatcggtcagtctgccgaccctctgagcagctggctggtcaactctgctcccttcatccgtgaccagctcaagttcctgacccagacctaccctgccaagggtggtatctacttctccgagttcggctgggcggaagatgcggaatacgaccgtcagctcctctaccagatcacctgggatggcctgcgcacccagtacctgaccgactacctcagccagctcctccttgccgttcacaaggatggcatcaacctgcgtggagcgttgacctggtcgttcgtcgacaactgggaatggggcttgggaatgcagcagaagttcggtttccagttcgtcaaccagtcggaccccgatctgacccgcaccttcaagctctccgcccacgcctacgctcagttcggccgcaaccacctg

SEQ ID NO: 4 - DNA, 1671 bp, Artificial Sequence
  sets out a codon-adapted DNA sequence for expression of SEQ ID NO: 2 in Aspergillus niger
atgatgctccacgctgccttgcttgttgctctcccctgcgttgttctcgccggtactgctgagctcgatgccctctggaacctggttgaagcgcagtaccccgtgcagactgctgctgtcaccactctcgtcaccgtccccgatgactacaagttcgaggccgaccctcctagctacgcccttgctggctacgagacttctgagatcgctggtctgaagttccccaagggtttcaagttcggtgttgctggtgctgctatccaggttgagggtgctgccaaggccgagggccgtggtcccagcacctgggactacctctgccaccactacgccagcacccagtgcaacaactacgaccccgatatcaccaccaaccactactacctgtaccctctggacttcgctcgcttacaacacctgggcatcaacacctactctttctccatcagctggactcgtatctacccccttggtgctggatacgtcaacgaggctggtcttgctcactacgatgccgtcatccactccgccaagaagtacggcttggagcctgttggtaccgtcttccactgggatactcctctttctctgatgctcaagtacggtgcctggcaggacactggtgaccagattgtgaaggacttcgtcacctacgccaccaccgtcttcaagcgttacggcaacgaggtcaagacctggttcaccttcaacgagcctcgtgtcttctgctcgcagaactccggtctgccctacaacttgacttaccccgagggtatcaactccacctccgccgtcttccgctgcacctacaacgtcctcaaggcccacggccacgccgtcaaggtctaccgtgatcttgttgcctccggtaccattgctgccggtgaaattggattcaagtcggatgacaactaccccatccctgctcgccccggcaacgccgatgatgaggagtctgccaagcgtcacgaagcgttccgcattggtatcttcgctcagcctgtctacggtaacggtgactaccccgatgttgtcaaggagactgtcggtgacatgcttcctgctctgaccgacgaggacaagggctacatcaagggttccggtgacatcttcgccatcgacggctaccgcactgacatctcccacgctgctctcaacggcattgccaactgcattcgcaaccagtccgaccccaactggcccgtctgcgaagaaggctccgaccccttcgctcacgtctacccctccggcttcgccattggccagtccgccgaccccctcagcagctggctggtcaactctgctcccttcatccgtgaccagctcaagttcctgacccagacctaccccgccaagggtggtatctacttctctgagttcggctgggctgaggatgccgagtacgaccgccagctcctctaccagatcacctgggatggtctgcgtacccagtacctgaccgactacctgtcccagctcctgctggccgtccacaaggatggcatcaacctccgtggtgccctcacctggtcgttcgtcgacaactgggaatggggtcttggcatgcagcagaagttcggtttccagttcgtcaaccagtcggatcctgacctcacccgcaccttcaagctctccgctcacgcctacgcccagttcggccgcaaccattta

SEQ ID NO: 5 - DNA, 13 bp, Artificial Sequence
  sets out the modified translational initiation sequence of the glucoamylase glaA promoter
caccgtcaaaatg

SEQ ID NO: 6 - DNA, 1998 bp, Artificial Sequence
  sets out the DNA fragments containing a.o. part of the glucoamylase promoter and the BHT-132 encoding gene including an EcoRI and PacI restriction site
gaattcaagctagatgctaagcgatattgcatggcaatatgtgttgatgcatgtgcttcttccttcagcttcccctcgtgcagatgaggtttggctataaattgaagtggttggtcggggttccgtgaggggctgaagtgcttcctcccttttagacgcaactgagagcctgagcttcatccccagcatcattacaccgtcaaaatgatgcttcacgctgctctccttgttgctcttccttgcgttgtccttgctcgtcccgccggtgctgtcacctaccccggtgccatccccctctccctcacctcgaactacgagactcccagccctactgccattcctctggagcccacccccactgccactggtactgctgagctcgatgccctctggaacttggttgaggctcagtaccccgtgcagactgctgccgtcaccaccctcgtcaccgttcccgatgactacaagttcgaggccgatcctcctagctacgctcttgctggatacgagacttctgagattgctggtctgaagttccccaagggcttcaagttcggtgttgctggtgccgccatccaggttgagggtgctgccaaggccgagggccgtggtccctccacctgggactacctctgccaccactacgcctccacccagtgcaacaactacgaccctgacatcaccaccaaccactactacctctaccccctcgacttcgctcgtctgcagcacctgggtatcaacacctactctttctccatctcctggactcgcatctaccctcttggtgctggctacgtcaacgaggctggtctggctcactacgatgccgtcatccactctgccaagaagtacggcttggagcctgttggtaccgtcttccactgggatactcctctgagcttgatgctcaagtacggtgcctggcaggacaccggtgaccagattgtcaaggacttcgtcacctacgccaccactgtcttcaagcgctacggcaacgaggtcaagacctggttcaccttcaacgagcctcgtgtcttctgctctcagaactccggtctgccctacaacctgacctacccagaaggcatcaactccacctcggcggtgttccgctgcacctacaacgtcctcaaggcccacggccacgccgtcaaggtctaccgtgatcttgttgcctccggtaccattgctgctggtgagatcggtttcaagtccgacgacaactaccccatccccgctcgccccggcaacgccgatgatgaggagtccgccaagcgtcacgaagcgttccgtatcggtatcttcgctcagcccgtgtatggcaacggtgactaccccgatgtcgtcaaggagactgttggtgacatgcttcccgccctcaccgacgaggacaagggctacatcaagggctccggtgacatcttcgccattgacggctaccgcactgatatatctcacgctgccctcaacggcattgccaactgcattcgcaaccagtccgaccccaactggcccgtctgcgaagaaggaagcgaccccttcgctcacgtctacccctccggattcgccatcggtcagtctgccgaccctctgagcagctggctggtcaactctgctcccttcatccgtgaccagctcaagttcctgacccagacctaccctgccaagggtggtatctacttctccgagttcggctgggcggaagatgcggaatacgaccgtcagctcctctaccagatcacctgggatggcctgcgcacccagtacctgaccgactacctcagccagctcctccttgccgttcacaaggatggcatcaacctgcgtggagcgttgacctggtcgttcgtcgacaactgggaatggggcttgggaatgcagcagaagttcggtttccagttcgtcaaccagtcggaccccgatctgacccgcaccttcaagctctccgcccacgcctacgctcagttcggccgcaaccacctgtaaattaattaa

SEQ ID NO: 7 - DNA, 1887 bp, Artificial Sequence
  sets out the DNA fragments containing a.o. part of the glucoamylase promoter and the BHT-134 encoding gene including an EcoRI and PacI restriction site
gaattcaagctagatgctaagcgatattgcatggcaatatgtgttgatgcatgtgcttcttccttcagcttcccctcgtgcagatgaggtttggctataaattgaagtggttggtcggggttccgtgaggggctgaagtgcttcctcccttttagacgcaactgagagcctgagcttcatccccagcatcattacaccgtcaaaatgatgctccacgctgccttgcttgttgctctcccctgcgttgttctcgccggtactgctgagctcgatgccctctggaacctggttgaagcgcagtaccccgtgcagactgctgctgtcaccactctcgtcaccgtccccgatgactacaagttcgaggccgaccctcctagctacgcccttgctggctacgagacttctgagatcgctggtctgaagttccccaagggtttcaagttcggtgttgctggtgctgctatccaggttgagggtgctgccaaggccgagggccgtggtcccagcacctgggactacctctgccaccactacgccagcacccagtgcaacaactacgaccccgatatcaccaccaaccactactacctgtaccctctggacttcgctcgcttacaacacctgggcatcaacacctactctttctccatcagctggactcgtatctacccccttggtgctggatacgtcaacgaggctggtcttgctcactacgatgccgtcatccactccgccaagaagtacggcttggagcctgttggtaccgtcttccactgggatactcctctttctctgatgctcaagtacggtgcctggcaggacactggtgaccagattgtgaaggacttcgtcacctacgccaccaccgtcttcaagcgttacggcaacgaggtcaagacctggttcaccttcaacgagcctcgtgtcttctgctcgcagaactccggtctgccctacaacttgacttaccccgagggtatcaactccacctccgccgtcttccgctgcacctacaacgtcctcaaggcccacggccacgccgtcaaggtctaccgtgatcttgttgcctccggtaccattgctgccggtgaaattggattcaagtcggatgacaactaccccatccctgctcgccccggcaacgccgatgatgaggagtctgccaagcgtcacgaagcgttccgcattggtatcttcgctcagcctgtctacggtaacggtgactaccccgatgttgtcaaggagactgtcggtgacatgcttcctgctctgaccgacgaggacaagggctacatcaagggttccggtgacatcttcgccatcgacggctaccgcactgacatctcccacgctgctctcaacggcattgccaactgcattcgcaaccagtccgaccccaactggcccgtctgcgaagaaggctccgaccccttcgctcacgtctacccctccggcttcgccattggccagtccgccgaccccctcagcagctggctggtcaactctgctcccttcatccgtgaccagctcaagttcctgacccagacctaccccgccaagggtggtatctacttctctgagttcggctgggctgaggatgccgagtacgaccgccagctcctctaccagatcacctgggatggtctgcgtacccagtacctgaccgactacctgtcccagctcctgctggccgtccacaaggatggcatcaacctccgtggtgccctcacctggtcgttcgtcgacaactgggaatggggtcttggcatgcagcagaagttcggtttccagttcgtcaaccagtcggatcctgacctcacccgcaccttcaagctctccgctcacgcctacgcccagttcggccgcaaccatttataaattaattaa